European Patent Application EP 4 353 078 A2, published April 17, 2024. Title: HELMINTHOSPORIUM TURCICUM-RESISTENTE PFLANZE. Applicant: KWS SAAT SE & Co. KGaA. Application EP. The sequence listing filed with the application follows.

SEQUENCE LISTING (250 sequences)

SEQ ID NO: 1 - DNA, 2004 bp, Zea mays
  source 1..2004: mol_type = other DNA
atggctgctcaccagcctcacctctccgtcctcctcctcgtcctcctcgctgcccatgtcgtctccacctccgcccatggcgagcctcctcttccgagcccttacaacacctccgcccatggcgagcctcctcttccgagcacttacaacgcctccatgtgctcgtcgttctggtgtggcggcgtcgagatccgctacccgttctatcttgccaacgcaatcgccgactacagcgggagctactactcctgcggctacaccgacttgagcgtttcctgcgaactcgaggtcgaggggtcgccgacgacctggacccctaccatccgtctcggcggcggcgactacaccgtcaagaacatctcctacctctacgaccagcagaccatctcactggcggacagagatgtgctcggaggcggcggctgccccgtcgtccgccacaacgtcagcttcgacgagacgtggctgcacctgcacaacgccagcgccttcgacaacctcaccttcttcttcggatgccactgggggccacggaatacaccgcctgaatttgccgactacaacatcagctgcgccgggttcaatactccaactatcagcggtggaaggtccttcgtgttcaagactggagatcttgacgaacaagaggagcaggagttggctttacactgcgacgaggttttctccgtgccagtgagaagagatgctctgcaggcgatcgtcagcaacttcagcctcacacgggacgggtacggcgaggtgcttaggcaggggttcgagttggaatggaatcggacatcggaggatcagtgtggccggtgcgagggatcgggctccggcggatggtgcgcctacagccagaagagagaattcctgggctgcttgtgcagcggagggaaggtgggcagcccgttctgcaaaccatcgagatcaaaaaggaaagaaggacctattgttggtgctgttgccgttgcattcctgtgtctagtcattctcacatgcttcttggcttgtagacatggttcgctgcccttcaaatcggagaacaaaccagggacaaggattgagtccttcctacagaagaacgagagtatacatccgaaaagatacacctacgcggacgtgaaaagaatgacaaaatccttcgctgtgaagctaggccaaggtgggtttggtgctgtatacaaaggcagcctccacgatggccgacaggtagcagtcaagatgctgaaggacacccaaggtgacggcgaggaattcatgaacgaggtggctagcatcagcaggacttctcatgtcaacgtcgtgacacttctagggttttgcttgcaagggtcgaaaagagcactgatctacgagtacatgcccaatggttcgctcgaaaggtatgccttcaccggtgacatgaacagtgagaatttgctaacctgggaaaggctatttgacatagcaattggcacggccagagggctcgaatacctacaccggggatgcaacactcggatcgtgcattttgacatcaagccacacaacatcctgttagaccaggatttctgtcctaagatctctgactttggactggccaagctatgtctgaacaaagagagcgctatctccattgctggcgcaagagggacgatagggtatatcgccccggaggtctactcaaagcaatttggaataataagcagcaagtctgatgtctatagctatgggatgatggtccttgagatggttggagcaagggacaggaatacaagcgcagatagtgaccatagcagccaatatttccctcagtggctttatgaacatttggacgactattgtgttggtgcttccgagattaatggtgagaccacagagctcgtgaggaagatgatagttgtaggtctgtggtgcatacaagtgattccgactgatcgaccaacaatgacgagagtcgtcgagatgttggaagggagcacaagtaatctagagttgccacccagagttctcttgagctga

SEQ ID NO: 2 - protein, 667 aa, Zea mays
MAAHQPHLSVLLLVLLAAHVVSTSAHGEPPLPSPYNTSAHGEPPLPSTYNASMCSSFWCGGVEIRYPFYLANAIADYSGSYYSCGYTDLSVSCELEVEGSPTTWTPTIRLGGGDYTVKNISYLYDQQTISLADRDVLGGGGCPVVRHNVSFDETWLHLHNASAFDNLTFFFGCHWGPRNTPPEFADYNISCAGFNTPTISGGRSFVFKTGDLDEQEEQELALHCDEVFSVPVRRDALQAIVSNFSLTRDGYGEVLRQGFELEWNRTSEDQCGRCEGSGSGGWCAYSQKREFLGCLCSGGKVGSPFCKPSRSKRKEGPIVGAVAVAFLCLVILTCFLACRHGSLPFKSENKPGTRIESFLQKNESIHPKRYTYADVKRMTKSFAVKLGQGGFGAVYKGSLHDGRQVAVKMLKDTQGDGEEFMNEVASISRTSHVNVVTLLGFCLQGSKRALIYEYMPNGSLERYAFTGDMNSENLLTWERLFDIAIGTARGLEYLHRGCNTRIVHFDIKPHNILLDQDFCPKISDFGLAKLCLNKESAISIAGARGTIGYIAPEVYSKQFGIISSKSDVYSYGMMVLEMVGARDRNTSADSDHSSQYFPQWLYEHLDDYCVGASEINGETTELVRKMIVVGLWCIQVIPTDRPTMTRVVEMLEGSTSNLELPPRVLLS

SEQ ID NO: 3 - DNA, 2133 bp, Zea mays
  source 1..2133: mol_type = other DNA
atggctgctcacctaccacgcctccccgtcctcctcctcgtcctcctcgctgcccatgtcgtctccacctccgcccatggcgagcctcctcttccgagcacttacaacacctccgcccatggcgagcctcttcttccgagcacttacaacgcctccatgtgctcggaatcgttctggtgtggcggcgtcgagatccgctacccgttcaatcttgccaacgcaaccgccgactacagcgggaactactactcctgcggctacaccgacttgagcgtttcctgcgaactcgaggtcgaagggtcgccgacgacctggacccctaccatccgtctcggcggcgacatctacaccgtcaagaacatctcctacgactatcataccatctcactggcggacaacgatgtgctcggaggcggcgagtgccccgtcgtccgccacaacgtcagcttcaacgagacgtggctgcacaacgccagcgccttcgacaacctcaccttcttcttcggatgccactgggggccacggaatacaccgcctgaatttgccgactacaacatcagctgcgccgggttcaatcctccaactatcagcggtggagactccttcgtgttcaagcctgaatatcttgacgaacaagaggagcaggagttggcttcacactgcgacgaggttttctccgtgccagtcagaagcgatgctctgcgggcgaccttcagcctcacagggtacgggtacggcgagctgcttaggcaggggttcgggttggaatggaatcggacatcggaggatcagtgtggccagtgcgagggatcgggctccggcggatggtgcgcctacagccagaagagagaattcctgggctgcttgtgcagcggagggaaggtgggcaacccgttctgcaaaccatcgaagtcaacaaggaaaccaagaattcttgctggtgccctgggtggtggtgctgctgcgctgcttgttggtgctgccatatttttgttcgtcatcatgcgcaagaggaagcagaagaagaaagtgaccaactcgtcttcgaagctcctcaagtacagcggctctggtgggaccccgcgttcgcgggttggtgacatggagtccggcagcatcgaggacccgccaacgcaccacttcgcctacgaggagctcgaggaggcgaccaaccgcttcgacgaaagcagagaactcggcgatggcggcttcggcaccgtctacaaagggtacctcagggacgggcgcgtggtggcggtgaagcggctgtacaacaacgggtaccggcgcgtggagcagttccagaacgaggcggccatcctgtcggggctgcgccacccaaacctcgtcatgttctacggctgcacgtccagccacagccgcgagctcctgctggtgtacgagttcgtggccaacggcacggtcgccgaccacctgcacgggcagcgggcccccgagcgcgccctctcgtggccgctccgcctcagcgtcgccgtggagtccgccgcggcgctcacctacctgcacgccatcgagccgcccgtcgtgcaccgcgacgtcaagaccaccaacatcctcctggacgccgactaccacgtcaaggtcgccgacttcggcctctcccgcctcttccccctcgacgtcacgcacgtctccaccgctccgcagggcacgccagggtatgttgatccagagtaccaccagtgctaccagctgacggacaagagcgacgtgtacagcttcggggtggtcctggtggagctcatctcgtccaagccggccgtcgacatcacccggcaccgcagcgagatcaacctggccagcatggccatcagcaagatccagaagtgccagctggaggagctcgtcgacctcggcctgggctacgacaccgacccggccaccaggaagatgatgacgatggtcgcggagctggccttccgctgcctgcagcagaacggcgagatgcgcccgccgatcaaggaggtgctcgaggtgctcaggaacatccagggcgagtgtctgacgtcggggaaggatggggacaagagcaaggacgggcccttctctcccaccacggttcacgctccgtgggacagcaggtccacgacgcccaacaccagcagggactag

SEQ ID NO: 4 - protein, 710 aa, Zea mays
MAAHLPRLPVLLLVLLAAHVVSTSAHGEPPLPSTYNTSAHGEPLLPSTYNASMCSESFWCGGVEIRYPFNLANATADYSGNYYSCGYTDLSVSCELEVEGSPTTWTPTIRLGGDIYTVKNISYDYHTISLADNDVLGGGECPVVRHNVSFNETWLHNASAFDNLTFFFGCHWGPRNTPPEFADYNISCAGFNPPTISGGDSFVFKPEYLDEQEEQELASHCDEVFSVPVRSDALRATFSLTGYGYGELLRQGFGLEWNRTSEDQCGQCEGSGSGGWCAYSQKREFLGCLCSGGKVGNPFCKPSKSTRKPRILAGALGGGAAALLVGAAIFLFVIMRKRKQKKKVTNSSSKLLKYSGSGGTPRSRVGDMESGSIEDPPTHHFAYEELEEATNRFDESRELGDGGFGTVYKGYLRDGRVVAVKRLYNNGYRRVEQFQNEAAILSGLRHPNLVMFYGCTSSHSRELLLVYEFVANGTVADHLHGQRAPERALSWPLRLSVAVESAAALTYLHAIEPPVVHRDVKTTNILLDADYHVKVADFGLSRLFPLDVTHVSTAPQGTPGYVDPEYHQCYQLTDKSDVYSFGVVLVELISSKPAVDITRHRSEINLASMAISKIQKCQLEELVDLGLGYDTDPATRKMMTMVAELAFRCLQQNGEMRPPIKEVLEVLRNIQGECLTSGKDGDKSKDGPFSPTTVHAPWDSRSTTPNTSRD

SEQ ID NO: 5 - DNA, 879 bp, Zea mays
  source 1..879: mol_type = other DNA
atggctcctctgctcctgctcctgctcctcttccccgtccagttccagctcctgctcctcctagccgtagccgacgctgtccccggtctctgcgccagagccacatgcgccggccatgtcatccagtacccgttctggctcaactcctcggcgcccgactgcggccgccgccacgggatcggccttgtctgcgagggcaactcgacgctgaccctcccctacatgtcccacagatacgtagtgtccagcatcgactacaagacgcgtaccgtgctggtctcggacgccgacatcggcgacgagtacgacgcggccggctgcccgcgcgtccgcgtgaacctcaccatcgacaccgcctggctgcggcccgcggcctccgacgccaacatcaccttcctctacgactgcaagaagagcatcaccctgccctccgccgtggaactgagtgggtgccattgccaccagcagcagcagcagcagcaacaggattattgccgtaggtcgtacgtgctgccggacggcgggatcacgggcgccgaggcgcaccagtacgggtgcgaggacgtggtggtggcgccggtgctggacgcgcacaggagggagatcctgggcgcgcctccggcgaacggatccctccgccgggtgctgcagggcgggttcgagctgaactacgacacccactctgagctgtgcgaccggtgcgaggcctccggcgggtggtgcggctaccggcgcggcgaggcgcccgccaccggcgccggcggcgggctgacgttcgcctgcttctgcgacggcggcccgacgacgacgggcctgtgcggtgccggtacgtacctcctcttcattcccccagcgttacaatttattatatgtttgtaa

SEQ ID NO: 6 - protein, 292 aa, Zea mays
MAPLLLLLLLFPVQFQLLLLLAVADAVPGLCARATCAGHVIQYPFWLNSSAPDCGRRHGIGLVCEGNSTLTLPYMSHRYVVSSIDYKTRTVLVSDADIGDEYDAAGCPRVRVNLTIDTAWLRPAASDANITFLYDCKKSITLPSAVELSGCHCHQQQQQQQQDYCRRSYVLPDGGITGAEAHQYGCEDVVVAPVLDAHRREILGAPPANGSLRRVLQGGFELNYDTHSELCDRCEASGGWCGYRRGEAPATGAGGGLTFACFCDGGPTTTGLCGAGTYLLFIPPALQFIICL

SEQ ID NO: 7 - DNA, 588 bp, Zea mays
  source 1..588: mol_type = other DNA
atggggtgcacgacctcccacgacgccgtcgccgctgctgtcacctcctccagttcccggccccgtgcgcgccgctcgtccgcgtccgacccctcaccacggcgcggagaccccgccgcgctgtgccgcgagcgcgtggcgctcatccacgccgcgaccgaccgccggtacgcgctcgccaccgcgcacgctgcctacttccgctcgctcgccgccgtcggtgacgcgctgcggcgcttcgtggcgtccgcgctcgcgcccgccacgcctgggtcctcgctggtgctcacgctcccgccttcccccgccaagctggtcgctgccgcgtccgccagcctcccgacgtggccgttgtccaccgtctcgtcgctctcgcactccctcgcagagaagcggcggatctttagggaggcggcgttgaagggaagcgcgcgagagaggacacagtcacggactcaggccaccgttgctcacagctgcattagaatccgatttcgggtccacgctcacacgtgtcaacgccggatacgggatgctaacgtgaagtgcggacgaggcttcaaaaggggtgaggttttaataacttag

SEQ ID NO: 8 - protein, 195 aa, Zea mays
MGCTTSHDAVAAAVTSSSSRPRARRSSASDPSPRRGDPAALCRERVALIHAATDRRYALATAHAAYFRSLAAVGDALRRFVASALAPATPGSSLVLTLPPSPAKLVAAASASLPTWPLSTVSSLSHSLAEKRRIFREAALKGSARERTQSRTQATVAHSCIRIRFRVHAHTCQRRIRDANVKCGRGFKRGEVLIT

SEQ ID NO: 9 - DNA, 3699 bp, Zea mays
  source 1..3699: mol_type = other DNA
atggcgacgccgacgcccatgcctggaggcgaggggacgctcgcagcggtgatgccgcggtccccgtctccgacgccggcggaggcggggacctcggcgaccgagacgcccgtgctgatattcctttactttcacaaggcgatccgcgcggagctcgaggcgctgcacggcgccgccgtgctcctggccaccgagcgcaccggcgatgtagagatgctcgccaagcgctgccgcttcttcttcaacatttacaaacaccactgcgacgccgaggatgcggtcatttttccagcactcgatatccgagtaaagaatgttgcagggacctattccttagagcataaaggagaaagcgatctttttagccagttatttgatctcctgcaattggacatacataatgatgatggtcttcgtagggagcttgcgtcatgcacaggcgcgatacagacatgtctcagccaacatatgtccaaggaggaagaacaggtctttccattgcttacaaagaaattttcgtgtgaagaacaagctgatttagtgtggcaattcctatgcaacattcctgtcaatatggtggcagagttccttccatggctttcaacttctgtcacatctgatgagcaccaagatatccgtaactgcttatgcaaagtagttcctgatgagaaacttctccaacaggttgtattcacatggatggaagggaaagcaacaagagaagtggcagagagcattgctgctggtatttcagcaagaaatcatagtgttgaggatgtcccagaccaagggaagattcatatttgtttacatcacaattctaaacttgggagtaaaaactgtggagaatctaatggtcctcaggctgacaagcatcctatagatgatattttatactggcacaatgctattcgtatggagttacgtgatataaaagaggagacaagaagggtgcagcaatctggggatttttctgatatatcagccttcaatgagaggcttcagttcattgcagatgtatgcatctaccacagtatcgctgaggatcaggttgtttttcctgcagtcgatagtgagctgtcctttgtgcaggagcatgctgaagaagaatgcaggtttaacaattttaggtgtttaattcagcaaatccaaatagcaggagccgaatcaactgcattggacttctactcaaaactgtgttcacatgctgataaaatattggaggcaatcgaaaaacacttctgcaatgaagaaaccaaggtgcttcctcaagctaggatgctcttctctcttgagaagcaaagggaactttcatacaaaagtttgtgtgttatgccattgaaattattggaacgtgttttgccgtggttggtgtcgaagctgagtgatgttcaggcaacttcatttcttcagaatatacgcttggcagcatcaccatctgaaactgcactggtcactcttatctctggttgggcatgcaaaggccgggataaatccaaagatggagaatatttatgcttaacatcaggtgcggcgagatgtctatcagatgatgtagatgatctgggaaaatgccgatcattctgtccatgtgcttcacccaacagctcagatctttctctgcagctacatactgagaatgattctaggccaggcaagcgaggaaaagatgcagtatctttttctcatactaatggaatctactgctctcaaactgctgacattgaagcaattccatgtagcaaaaaaccatgttgtattcctggtttgagagtagagagtagcaatcttggtattggttccttggcttctgcaaagtcttttcactctttatcatacaattcaactgctccttcactatattcgagcctcttttcatgggagacagatacatcattgtcttgttcggacagcatttcaaggccaatcgatacaatattcaaatttcataaggcaattcgcaaggatttagaatacttagatgttgaatctggcaagctcattgatggcaacgagtcctgccttcgccaattcattggaaggttccgtttgttatggggtctttacagggctcacagcaatgctgaggatgaaattgtgtttccagcattggaatccagagaaacattacacaatgtgagccattcatatactcttgaccacaagcaggaagaacagttgtttgaagatatctcaaatgttctctttcaactttcacaactacatgatagccagggccatgcccagactgaagttaatgaagtaaagaaaagctgtttccattcatctaatgatgtcgattttgctagaaagtataatgaacttgccacaaaacttcagggcatgtgcaagtctatccgggtcgccttgactaatcatgtccatagagaagaacttgaattatggccgttgtttgataaacatttttctgtggaggagcaagataaacttgtaggtcgtataattggttcaacaggtgctgaggttctccaatctatgttaccctgggttacatcagttctcactcaagaggagcagaacaaaatgcttgatatgtggaagcaagctacaaaaaatacaatgtttggggaatggctaaacgagtggtggaagggagctggaacagcatctgattcttcagcagaggcgtcctctgctccagaagatagtcatttacaagataagcttgaacaaaatgaccagatgttcaagcctggctggaaggacatatttcgaatgaatcagagtgaacttgaggctgaggtgcgaaaggtttcacgagattctacacttgacccaaggcggaaggcgtatctaattcaaaatctcatgacaagccgctggatagctgcacagcagaagttaccagaaccaaattctgaagaatgtaatcacgatgccagtatacctggatgtgcaccttcataccgagaccaggagaaacaaatttatggttgtgaacactacaaacggaactgcaaacttgttgctgcatgctgcaacaagctcttcacatgcaggttctgccatgataaagttagtgaccatacgatggaaaggaaagcaacacaggagatgatgtgcatggtatgcctaaagattcaacctgttggttcgttctgccaaaccccatcttgcaacagactatcgatggcaaagtactactgtaacatctgtaaattttttgatgatgaaaggactgtgtaccactgtccgttttgtaatttgtgtcgtcttgggaaaggtcttggtgttgatttcttccattgcatgaaatgcaactgctgccttggaatgaaattaactgagcacaaatgtcgggaaaaagggctagagacaaattgtccaatatgctgtgacttcctatttacatcaagtgccgcagtcagagccctcccttgtggccacttcatgcattcagcttgctttcaggcatacacttgtagtcactacacttgccctatctgctgcaaatccttgggagatatggcggtttattttggcatgcttgatgccttgttggcggctgaagagcttccggaggaataccgtgatcggtgtcaggatatactttgcaatgactgtgagaggaaaggtagatgtcgatttcattggttataccacaaatgcggctcctgtgggtcgtacaacacccgagttatcaagactgccacagcagattgctctacaccaaactag

SEQ ID NO: 10 - protein, 1232 aa, Zea mays
MATPTPMPGGEGTLAAVMPRSPSPTPAEAGTSATETPVLIFLYFHKAIRAELEALHGAAVLLATERTGDVEMLAKRCRFFFNIYKHHCDAEDAVIFPALDIRVKNVAGTYSLEHKGESDLFSQLFDLLQLDIHNDDGLRRELASCTGAIQTCLSQHMSKEEEQVFPLLTKKFSCEEQADLVWQFLCNIPVNMVAEFLPWLSTSVTSDEHQDIRNCLCKVVPDEKLLQQVVFTWMEGKATREVAESIAAGISARNHSVEDVPDQGKIHICLHHNSKLGSKNCGESNGPQADKHPIDDILYWHNAIRMELRDIKEETRRVQQSGDFSDISAFNERLQFIADVCIYHSIAEDQVVFPAVDSELSFVQEHAEEECRFNNFRCLIQQIQIAGAESTALDFYSKLCSHADKILEAIEKHFCNEETKVLPQARMLFSLEKQRELSYKSLCVMPLKLLERVLPWLVSKLSDVQATSFLQNIRLAASPSETALVTLISGWACKGRDKSKDGEYLCLTSGAARCLSDDVDDLGKCRSFCPCASPNSSDLSLQLHTENDSRPGKRGKDAVSFSHTNGIYCSQTADIEAIPCSKKPCCIPGLRVESSNLGIGSLASAKSFHSLSYNSTAPSLYSSLFSWETDTSLSCSDSISRPIDTIFKFHKAIRKDLEYLDVESGKLIDGNESCLRQFIGRFRLLWGLYRAHSNAEDEIVFPALESRETLHNVSHSYTLDHKQEEQLFEDISNVLFQLSQLHDSQGHAQTEVNEVKKSCFHSSNDVDFARKYNELATKLQGMCKSIRVALTNHVHREELELWPLFDKHFSVEEQDKLVGRIIGSTGAEVLQSMLPWVTSVLTQEEQNKMLDMWKQATKNTMFGEWLNEWWKGAGTASDSSAEASSAPEDSHLQDKLEQNDQMFKPGWKDIFRMNQSELEAEVRKVSRDSTLDPRRKAYLIQNLMTSRWIAAQQKLPEPNSEECNHDASIPGCAPSYRDQEKQIYGCEHYKRNCKLVAACCNKLFTCRFCHDKVSDHTMERKATQEMMCMVCLKIQPVGSFCQTPSCNRLSMAKYYCNICKFFDDERTVYHCPFCNLCRLGKGLGVDFFHCMKCNCCLGMKLTEHKCREKGLETNCPICCDFLFTSSAAVRALPCGHFMHSACFQAYTCSHYTCPICCKSLGDMAVYFGMLDALLAAEELPEEYRDRCQDILCNDCERKGRCRFHWLYHKCGSCGSYNTRVIKTATADCSTPN

SEQ ID NO: 11 - DNA, 1152 bp, Zea mays
  source 1..1152: mol_type = other DNA
atggagagctgggtccgcgcggtggtggaggccatccactcctctcgctcccagacagtcatctacctcgccggcggtgcatcccaggcgctcggttggctcctctccgtgcccggcgcttcgggcaccgtcctcgaggtcgtcgtgccctactctagggcctccatggcgcagctccttggcaagatgcccctgcaattcactagcaagcaggctgcagaggacatggcactggccgcatacaatcgagcactcaagctttctggaccaggtctgcaagttatgggtgttggatttactgggtcactggcgagctcacgtccaaaacatggtgaccacaggttttatgtgtcaacatggacacataattgtctcaggacatcacatgttaccttgtcgaagggtttacggagtagggaggaagaagacaaggtttcaagctactttttgcttaaggcaatagcagatacctgcagagtttctgcaaccattcagccagacattcacaaatctgaaattccagaagaaatcatggaacaatttgatgaagatcaagaactccagcaagttattaatgggcaagtttgcatgaaagtatataattttgctgctccggcggaaagtaacttgaacagaaaaataattctgcctggttcgttcaaccccttgcacgatggtcaccttagattgctagaagctgcagtaagcatgtgtgatgatgggcttccattctttgagatatcagcaattaatgctgataaacctccactatctattgcagaaattaagaggcgtgttgagcaatttagaaaagcagggaagaatgtgattatatctaaccagccatacttctataagaaagcagaacttttcccaggaagcgcttttataattggtgcagacactgcagcaaggcttgttaaccctaagtactatggaggagattacaacagaatgctggagatacttctcgaatgtaagagcatagggactacttttcttgttggtggtcgaaagattgaaggagatttcaaggtccttgagaacttagacattccagaagagctgagagaaatgttcatttctattccggaggaaaagtttcgcatagatatttcatctactgaaataagaaagagccaagggctctga

SEQ ID NO: 12 - protein, 383 aa, Zea mays
MESWVRAVVEAIHSSRSQTVIYLAGGASQALGWLLSVPGASGTVLEVVVPYSRASMAQLLGKMPLQFTSKQAAEDMALAAYNRALKLSGPGLQVMGVGFTGSLASSRPKHGDHRFYVSTWTHNCLRTSHVTLSKGLRSREEEDKVSSYFLLKAIADTCRVSATIQPDIHKSEIPEEIMEQFDEDQELQQVINGQVCMKVYNFAAPAESNLNRKIILPGSFNPLHDGHLRLLEAAVSMCDDGLPFFEISAINADKPPLSIAEIKRRVEQFRKAGKNVIISNQPYFYKKAELFPGSAFIIGADTAARLVNPKYYGGDYNRMLEILLECKSIGTTFLVGGRKIEGDFKVLENLDIPEELREMFISIPEEKFRIDISSTEIRKSQGL

SEQ ID NO: 13 - DNA, 666 bp, Zea mays
  source 1..666: mol_type = other DNA
atgcaccctaattttccaagcgatcatggcaacggacgaggggtgggcggcggcggcggccatagcaggcgcaagccgattcatcagcttctcggtggagggcgagccgcggacatcttgctgtggaaggacaggaatttgtctgcaggcctgctcgctggggccacgctggtatggtacctgttcgaggttgttgagtacagcattgtaccgctcgtttgccagatagccatcctggccatgctcgtcgtcttcatctggtcgaatgctgcgcccctcttgaacatagcccctccaaggatcccagaagtgatcatctctgagcatgccttccgacaaatagcacagatcgtccattacaaactggcacacaccgtgtctgctctttatgacattgcatgcgggaaggatctgaagaaattcctcctggtggtcttatcactgctaatagtgtcagaggttggaagttcttacagcttcacaagtcttctatatcttggatttctttgcgcccacactttgccagcgttgtaccaaagatatgagacagaggttgaccaccttgccgcaaggggtagtgaagacatcaagaggttctacaagaggattgattccaatttgctgaacaaaataccaaggggcccagtcaagacaaaagttaaataa

SEQ ID NO: 14 - protein, 221 aa, Zea mays
MHPNFPSDHGNGRGVGGGGGHSRRKPIHQLLGGGRAADILLWKDRNLSAGLLAGATLVWYLFEVVEYSIVPLVCQIAILAMLVVFIWSNAAPLLNIAPPRIPEVIISEHAFRQIAQIVHYKLAHTVSALYDIACGKDLKKFLLVVLSLLIVSEVGSSYSFTSLLYLGFLCAHTLPALYQRYETEVDHLAARGSEDIKRFYKRIDSNLLNKIPRGPVKTKVK

SEQ ID NO: 15 - DNA, 1113 bp, Zea mays
  source 1..1113: mol_type = other DNA
atgggcggcgtcacgtccaccatcgccgcgcgcttcgccttcttcccgccgacgccgccgtcctacaccgtcgtcgtcgccgacgccgccaccggtcgcctcgccatcccggagatctcccgggcaccctcgcgccgtcggaggcgggacggcgccggcgccgggggctcctcctcggcctcctccgtcgtcgcggccgccgaggaggaggacggcgcggaggtggtgcgcctccggacccgccgcgggaacgagatcgtgggggtctacgtgcgccacgcgcgggcctccgccaccgtgctctactcccacggcaacgccgccgacctcggccagatgtacgggctcttcgtcgagctcagccgccgcctccgcgtcaacctctttgggtatgattattctggttatgggagatctacagggaagcccactgagtgtaatacatatgcagacattgaagcagcatataactgcctcaaggaaaaatatggtgtagcagatgaggatataatcttatatggtcagtctgttggaagtggtccaaccattgatcttgcttcgcggttgccagacttgcgagctgtggttttgcatagtcctattttatctggactaagagtaatatatccagtcaagcggacgttttggtttgacatttacaagaacatcgataaaattggcttggtaaattgtccggtgcttgtcattcatggtacatcagatgacgtggttgactgctcccacggaaaacagctatgggagcactgcaaagtaaaatattctccactgtggttaagtggtggtggccactgcaatctcgagctatatccagattacattaagcacttgaaaaagtttgtgtcaagcgttagcaaaaaagcatcatcgaaacctgacccaaaagaaacaacgacaaaggatgacactaccagtaaagaaacagaggaagcgtacccggagaaacctcaagaggccaagaagtgcccgcagatctcgcgaaagagcctggacagccgattcgggaaatccaaaacagtggatgttcctgataaaccacggatgagctcggacgacatcgacaagttccggaggagcagatgcttggtctggtga

SEQ ID NO: 16 - protein, 370 aa, Zea mays
MGGVTSTIAARFAFFPPTPPSYTVVVADAATGRLAIPEISRAPSRRRRRDGAGAGGSSSASSVVAAAEEEDGAEVVRLRTRRGNEIVGVYVRHARASATVLYSHGNAADLGQMYGLFVELSRRLRVNLFGYDYSGYGRSTGKPTECNTYADIEAAYNCLKEKYGVADEDIILYGQSVGSGPTIDLASRLPDLRAVVLHSPILSGLRVIYPVKRTFWFDIYKNIDKIGLVNCPVLVIHGTSDDVVDCSHGKQLWEHCKVKYSPLWLSGGGHCNLELYPDYIKHLKKFVSSVSKKASSKPDPKETTTKDDTTSKETEEAYPEKPQEAKKCPQISRKSLDSRFGKSKTVDVPDKPRMSSDDIDKFRRSRCLVW

SEQ ID NO: 17 - DNA, 47 bp, synthetic construct
  misc_feature 1..47: note = SYN14136 Primer Allel X
  source 1..47: mol_type = other DNA
gaaggtgaccaagttcatgctcatcttgttcggccttttctacacta

SEQ ID NO: 18 - DNA, 46 bp, synthetic construct
  misc_feature 1..46: note = SYN14136 Primer Allel Y
  source 1..46: mol_type = other DNA
gaaggtcggagtcaacggattatcttgttcggccttttctacactc

SEQ ID NO: 19 - DNA, 28 bp, synthetic construct
  misc_feature 1..28: note = SYN14136 gemeinsamer Primer
  source 1..28: mol_type = other DNA
agaaccaaaaattcaccagctgtgagaa

SEQ ID NO: 20 - DNA, 44 bp, synthetic construct
  misc_feature 1..44: note = PZE-108076510 Primer Allel X
  source 1..44: mol_type = other DNA
gaaggtgaccaagttcatgctagcggcgggctttcatacaattt

SEQ ID NO: 21 - DNA, 43 bp, synthetic construct
  misc_feature 1..43: note = PZE-108076510 Primer Allel Y
  source 1..43: mol_type = other DNA
gaaggtcggagtcaacggattgcggcgggctttcatacaattc

SEQ ID NO: 22 - DNA, 24 bp, synthetic construct
  misc_feature 1..24: note = PZE-108076510 gemeinsamer Primer
  source 1..24: mol_type = other DNA
cttgtgatcacgtgaggggctcaa

SEQ ID NO: 23 - DNA, 49 bp, synthetic construct
  misc_feature 1..49: note = SYN24931 Primer Allel X
  source 1..49: mol_type = other DNA
gaaggtgaccaagttcatgctccattagatgagaaagcaaagagaacta

SEQ ID NO: 24 - DNA, 48 bp, synthetic construct
  misc_feature 1..48: note = SYN24931 Primer Allel Y
  source 1..48: mol_type = other DNA
gaaggtcggagtcaacggattcattagatgagaaagcaaagagaactg

SEQ ID NO: 25 - DNA, 25 bp, synthetic construct
  misc_feature 1..25: note = SYN24931 gemeinsamer Primer
  source 1..25: mol_type = other DNA
attggtcgacatctcatggaggctt

SEQ ID NO: 26 - DNA, 36 bp, synthetic construct
  misc_feature 1..36: note = PZE-108077560 Primer Allel X
  source 1..36: mol_type = other DNA
gaaggtgaccaagttcatgctgcagtggcctgcgca

SEQ ID NO: 27 - DNA, 39 bp, synthetic construct
  misc_feature 1..39: note = PZE-108077560 Primer Allel Y
  source 1..39: mol_type = other DNA
gaaggtcggagtcaacggattgctgcagtggcctgcgcg

SEQ ID NO: 28 - DNA, 28 bp, synthetic construct
  misc_feature 1..28: note = PZE-108077560 gemeinsamer Primer
  source 1..28: mol_type = other DNA
agataatgagtcatcaggctatcagcaa

SEQ ID NO: 29 - DNA, 49 bp, synthetic construct
  misc_feature 1..49: note = PZE-108093423 Primer Allel X
  source 1..49: mol_type = other DNA
gaaggtgaccaagttcatgctgtaatccattgtgaacatatcgctatca

SEQ ID NO: 30 - DNA, 47 bp, synthetic construct
  misc_feature 1..47: note = PZE-108093423 Primer Allel Y
  source 1..47: mol_type = other DNA
gaaggtcggagtcaacggattaatccattgtgaacatatcgctatcg

SEQ ID NO: 31 - DNA, 25 bp, synthetic construct
  misc_feature 1..25: note = PZE-108093423 gemeinsamer Primer
  source 1..25: mol_type = other DNA
gaaacggttctgctgcagtttggta

SEQ ID NO: 32 - DNA, 47 bp, synthetic construct
  misc_feature 1..47: note = PZE-108093748 Primer Allel X
  source 1..47: mol_type = other DNA
gaaggtgaccaagttcatgctggatagagttgcagctaatgcttcaa

SEQ ID NO: 33 - DNA, 46 bp, synthetic construct
  misc_feature 1..46: note = PZE-108093748 Primer Allel Y
  source 1..46: mol_type = other DNA
gaaggtcggagtcaacggattgatagagttgcagctaatgcttcag

SEQ ID NO: 34 - DNA, 28 bp, synthetic construct
  misc_feature 1..28: note = PZE-108093748 gemeinsamer Primer
  source 1..28: mol_type = other DNA
cctgcgctttgtaaataagttaggcaaa

SEQ ID NO: 35 - DNA, 38 bp, synthetic construct
  misc_feature 1..38: note = PZE-108107671 Primer Allel X
  source 1..38: mol_type = other DNA
gaaggtgaccaagttcatgcttgcacctgcacacgccg

SEQ ID NO: 36 - DNA, 40 bp, synthetic construct
  misc_feature 1..40: note = PZE-108107671 Primer Allel Y
  source 1..40: mol_type = other DNA
gaaggtcggagtcaacggattcttgcacctgcacacgccc

SEQ ID NO: 37 - DNA, 21 bp, synthetic construct
  misc_feature 1..21: note = PZE-108107671 gemeinsamer Primer
  source 1..21: mol_type = other DNA
gatgccaaggatcgggcgctt

SEQ ID NO: 38 - DNA, 47 bp, synthetic construct
  misc_feature 1..47: note = SYN4196 Primer Allel X
  source 1..47: mol_type = other DNA
gaaggtgaccaagttcatgctctgcactctggaatatctataacaga

SEQ ID NO: 39 - DNA, 47 bp, synthetic construct
  misc_feature 1..47: note = SYN4196 Primer Allel Y
  source 1..47: mol_type = other DNA
gaaggtcggagtcaacggattctgcactctggaatatctataacagc

SEQ ID NO: 40 - DNA, 25 bp, synthetic construct
  misc_feature 1..25: note = SYN4196 gemeinsamer Primer
  source 1..25: mol_type = other DNA
tggtttataccaggaagggacgcat

SEQ ID NO: 41 - DNA, 41 bp, synthetic construct
  misc_feature 1..41: note = MA0004 Primer Allel X
  source 1..41: mol_type = other DNA
gaaggtgaccaagttcatgctgcctcgtccgcacttcacgt

SEQ ID NO: 42 - DNA, 40 bp, synthetic construct
  misc_feature 1..40: note = MA0004 Primer Allel Y
  source 1..40: mol_type = other DNA
gaaggtcggagtcaacggattcctcgtccgcacttcacgg

SEQ ID NO: 43 - DNA, 22 bp, synthetic construct
  misc_feature 1..22: note = MA0004 gemeinsamer Primer
  source 1..22: mol_type = other DNA
gtgtcaacgccggatacgggat

SEQ ID NO: 44 - DNA, 52 bp, synthetic construct
  misc_feature 1..52: note = MA0005 Primer Allel X
  source 1..52: mol_type = other DNA
gaaggtgaccaagttcatgctccaaaattttagaatcacaaacagatttacg

SEQ ID NO: 45 - DNA, 52 bp, synthetic construct
  misc_feature 1..52: note = MA0005 Primer Allel Y
  source 1..52: mol_type = other DNA
gaaggtcggagtcaacggattccaaaattttagaatcacaaacagatttact

SEQ ID NO: 46 - DNA, 30 bp, synthetic construct
  misc_feature 1..30: note = MA0005 gemeinsamer Primer
  source 1..30: mol_type = other DNA
aaacgccagtatcaaggagttattagtatt

SEQ ID NO: 47 - DNA, 49 bp, synthetic construct
  misc_feature 1..49: note = MA0006 Primer Allel X
  source 1..49: mol_type = other DNA
gaaggtgaccaagttcatgctgcacacaaacacaaattatgtcaaactg

SEQ ID NO: 48 - DNA, 50 bp, synthetic construct
  misc_feature 1..50: note = MA0006 Primer Allel Y
  source 1..50: mol_type = other DNA
gaaggtcggagtcaacggattagcacacaaacacaaattatgtcaaacta

SEQ ID NO: 49 - DNA, 29 bp, synthetic construct
  misc_feature 1..29: note = MA0006 gemeinsamer Primer
  source 1..29: mol_type = other DNA
ggctgtcttacgatataccagttttctta

SEQ ID NO: 50 - DNA, 43 bp, synthetic construct
  misc_feature 1..43: note = PZE-108097482 Primer Allel X
  source 1..43: mol_type = other DNA
gaaggtgaccaagttcatgctagtcggggatgcatgccattga

SEQ ID NO: 51 - DNA, 42 bp, synthetic construct
  misc_feature 1..42: note = PZE-108097482 Primer Allel Y
  source 1..42: mol_type = other DNA
gaaggtcggagtcaacggattgtcggggatgcatgccattgc

SEQ ID NO: 52 - DNA, 25 bp, synthetic construct
  misc_feature 1..25: note = PZE-108097482 gemeinsamer Primer
  source 1..25: mol_type = other DNA
gactccagagagagacagaaaggaa

SEQ ID NO: 53 - DNA, 41 bp, synthetic construct; identical to SEQ ID NO: 41
  misc_feature 1..41: note = MA0002 Primer Allel X
  source 1..41: mol_type = other DNA

SEQ ID NO: 54 - DNA, 40 bp, synthetic construct; identical to SEQ ID NO: 42
  misc_feature 1..40: note = MA0002 Primer Allel Y
  source 1..40: mol_type = other DNA

SEQ ID NO: 55 - DNA, 22 bp, synthetic construct
  misc_feature 1..22: note = MA0002 gemeinsamer Primer
  source 1..22: mol_type = other DNA
gtgtcaacgccggatacgggat

SEQ ID NO: 56 - DNA, 41 bp, synthetic construct
  misc_feature 1..41: note = MA0003 Primer Allel X
  source 1..41: mol_type = other DNA
gaaggtgaccaagttcatgctccgtgatgcgccttgccgta

SEQ ID NO: 57 - DNA, 40 bp, synthetic construct
  misc_feature 1..40: note = MA0003 Primer Allel Y
  source 1..40: mol_type = other DNA
gaaggtcggagtcaacggattcgtgatgcgccttgccgtc

SEQ ID NO: 58 - DNA, 24 bp, synthetic construct
  misc_feature 1..24: note = MA0003 gemeinsamer Primer
  source 1..24: mol_type = other DNA
gcacatcaatcgactcagccctat

SEQ ID NO: 59 - DNA, 48 bp, synthetic construct
  misc_feature 1..48: note = MA0007 Primer Allel X
  source 1..48: mol_type = other DNA
gaaggtgaccaagttcatgctgaaattattctcagcgagcatataacc

SEQ ID NO: 60 - DNA, 49 bp, synthetic construct
  misc_feature 1..49: note = MA0007 Primer Allel Y
  source 1..49: mol_type = other DNA
gaaggtcggagtcaacggattggaaattattctcagcgagcatataact

SEQ ID NO: 61 - DNA, 24 bp, synthetic construct
  misc_feature 1..24: note = MA0007 gemeinsamer Primer
  source 1..24: mol_type = other DNA
cgaacaggcagrcccatatgcttt

SEQ ID NO: 62 - DNA, 48 bp, synthetic construct
  misc_feature 1..48: note = MA0008 Primer Allel X
  source 1..48: mol_type = other DNA
gaaggtgaccaagttcatgctggtaaaatgaagtaaaagcatatgggc

SEQ ID NO: 63 - DNA, 50 bp, synthetic construct
  misc_feature 1..50: note = MA0008 Primer Allel Y
  source 1..50: mol_type = other DNA
gaaggtcggagtcaacggattgaggtaaaatgaagtaaaagcatatgggt

SEQ ID NO: 64 - DNA, 25 bp, synthetic construct
  misc_feature 1..25: note = MA0008 gemeinsamer Primer
  source 1..25: mol_type = other DNA
tagacggagggtgtacttatgcgaa

SEQ ID NO: 65 - DNA, 51 bp, synthetic construct
  misc_feature 1..51: note = MA0009 Primer Allel X
  source 1..51: mol_type = other DNA
gaaggtgaccaagttcatgctgtaacaaatttgtgctttatgtttctggtt

SEQ ID NO: 66 - DNA, 49 bp, synthetic construct
  misc_feature 1..49: note = MA0009 Primer Allel Y
  source 1..49: mol_type = other DNA
gaaggtcggagtcaacggattaacaaatttgtgctttatgtttctggtg

SEQ ID NO: 67 - DNA, 29 bp, synthetic construct
  misc_feature 1..29: note = MA0009 gemeinsamer Primer
  source 1..29: mol_type = other DNA
gatttsagcaagattaagctgattcacgt

SEQ ID NO: 68 - DNA, 47 bp, synthetic construct
  misc_feature 1..47: note = MA0010 Primer Allel X
  source 1..47: mol_type = other DNA
gaaggtgaccaagttcatgctgttggtaagagcctatagtcaataca

SEQ ID NO: 69 - DNA, 47 bp, synthetic construct
  misc_feature 1..47: note = MA0010 Primer Allel Y
  source 1..47: mol_type = other DNA
gaaggtcggagtcaacggattgttggtaagagcctatagtcaatacc

SEQ ID NO: 70 - DNA, 30 bp, synthetic construct
  misc_feature 1..30: note = MA0010 gemeinsamer Primer
  source 1..30: mol_type = other DNA
aattcatcayatgcttttcttctgctcttt

SEQ ID NO: 71 - DNA, 44 bp, synthetic construct
  misc_feature 1..44: note = MA0011 Primer Allel X
  source 1..44: mol_type = other DNA
gaaggtgaccaagttcatgctccttcctacagaagaacgagagc

SEQ ID NO: 72 - DNA, 44 bp, synthetic construct
  misc_feature 1..44: note = MA0011 Primer Allel Y
  source 1..44: mol_type = other DNA
gaaggtcggagtcaacggattccttcctacagaagaacgagagt

SEQ ID NO: 73 - DNA, 25 bp, synthetic construct
  misc_feature 1..25: note = MA0011 gemeinsamer Primer
  source 1..25: mol_type = other DNA
ttcacgtccgcgtaggtgtatcttt

SEQ ID NO: 74 - DNA, 47 bp, synthetic construct
  misc_feature 1..47: note = MA0012 Primer Allel X
  source 1..47: mol_type = other DNA
gaaggtgaccaagttcatgctatagacatcagacttgctgcttattg

SEQ ID NO: 75 - DNA, 49 bp, synthetic construct
  misc_feature 1..49: note = MA0012 Primer Allel Y
  source 1..49: mol_type = other DNA
gaaggtcggagtcaacggattctatagacatcagacttgctgcttatta

SEQ ID NO: 76 - DNA, 25 bp, synthetic construct
  misc_feature 1..25: note = MA0012 gemeinsamer Primer
  source 1..25: mol_type = other DNA
cccggaggtctactcaaagcaattt

SEQ ID NO: 77 - DNA, 45 bp, synthetic construct
  misc_feature 1..45: note = MA0013 Primer Allel X
  source 1..45: mol_type = other DNA
gaaggtgaccaagttcatgctccttccgacaaatagcacagatca

SEQ ID NO: 78 - DNA, 44 bp, synthetic construct
  misc_feature 1..44: note = MA0013 Primer Allel Y
  source 1..44: mol_type = other DNA
gaaggtcggagtcaacggattcttccgacaaatagcacagatcg

SEQ ID NO: 79 - DNA, 25 bp, synthetic construct
  misc_feature 1..25: note = MA0013 gemeinsamer Primer
  source 1..25: mol_type = other DNA
gacacggtgtgtgccagtttgtaat

SEQ ID NO: 80 - DNA, 47 bp, synthetic construct
  misc_feature 1..47: note = MA0014 Primer Allel X
  source 1..47: mol_type = other DNA
gaaggtgaccaagttcatgctcaacctctgacactattagcagtgat

SEQ ID NO: 81 - DNA, 46 bp, synthetic construct
  misc_feature 1..46: note = MA0014 Primer Allel Y
  source 1..46: mol_type = other DNA
gaaggtcggagtcaacggattaacctctgacactattagcagtgac

SEQ ID NO: 82 - DNA, 29 bp, synthetic construct
  misc_feature 1..29: note = MA0014 gemeinsamer Primer
  source 1..29: mol_type = other DNA
tgttctgtttctgattctaaggtggtctt

SEQ ID NO: 83 - DNA, 44 bp, synthetic construct
  misc_feature 1..44: note = MA0015 Primer Allel X
  source 1..44: mol_type = other DNA
gaaggtgaccaagttcatgctacaggtatgccttgctcataagc

SEQ ID NO: 84 - DNA, 45 bp, synthetic construct
  misc_feature 1..45: note = MA0015 Primer Allel Y
  source 1..45: mol_type = other DNA
gaaggtcggagtcaacggattcacaggtatgccttgctcataaga

SEQ ID NO: 85 - DNA, 26 bp, synthetic construct
  misc_feature 1..26: note = MA0015 gemeinsamer Primer
  source 1..26: mol_type = other DNA
catarccactgttctaggctggtgaa

SEQ ID NO: 86 - DNA, 43 bp, synthetic construct
  misc_feature 1..43: note = MA0016 Primer Allel X
  source 1..43: mol_type = other DNA
gaaggtgaccaagttcatgctcgagcaaccggagataaccaca

SEQ ID NO: 87 - DNA, 42 bp, synthetic construct
  misc_feature 1..42: note = MA0016 Primer Allel Y
  source 1..42: mol_type = other DNA
gaaggtcggagtcaacggattgagcaaccggagataaccacg

SEQ ID NO: 88 - DNA, 30 bp, synthetic construct
  misc_feature 1..30: note = MA0016 gemeinsamer Primer
  source 1..30: mol_type = other DNA
tttcggtaacttgagacctctaattctttt

SEQ ID NO: 89 - DNA, 38 bp, synthetic construct
  misc_feature 1..38: note = MA0017 Primer Allel X
  source 1..38: mol_type = other DNA
gaaggtgaccaagttcatgctcccaaacacgtcgcacg

SEQ ID NO: 90 - DNA, 43 bp, synthetic construct
  misc_feature 1..43: note = MA0017 Primer Allel Y
  source 1..43: mol_type = other DNA
gaaggtcggagtcaacggattatgctcccaaacacgtcgcaca

SEQ ID NO: 91 - DNA, 23 bp, synthetic construct
  misc_feature 1..23: note = MA0017 gemeinsamer Primer
  source 1..23: mol_type = other DNA
cgcccgtcacctaacaacagcaa

SEQ ID NO: 92 - DNA, 50 bp, synthetic construct
  misc_feature 1..50: note = MA0018 Primer Allel X
  source 1..50: mol_type = other DNA
gaaggtgaccaagttcatgctattctagagtatagatgtctaaacaaacc

SEQ ID NO: 93 - DNA, 47 bp, synthetic construct
  misc_feature 1..47: note = MA0018 Primer Allel Y
  source 1..47: mol_type = other DNA
gaaggtcggagtcaacggattctagagtatagatgtctaaacaaact

SEQ ID NO: 94 - DNA, 22 bp, synthetic construct
  misc_feature 1..22: note = MA0018 gemeinsamer Primer
  source 1..22: mol_type = other DNA
cgacgggtgacgagtgacgatt

SEQ ID NO: 95 - DNA, 46 bp, synthetic construct
  misc_feature 1..46: note = MA0019 Primer Allel X
  source 1..46: mol_type = other DNA
gaaggtgaccaagttcatgctataaatatctactcggcgccaatac

SEQ ID NO: 96 - DNA, 46 bp, synthetic construct
  misc_feature 1..46: note = MA0019 Primer Allel Y
  source 1..46: mol_type = other DNA
gaaggtcggagtcaacggattataaatatctactcggcgccaatag

SEQ ID NO: 97 - DNA, 27 bp, synthetic construct
  misc_feature 1..27: note = MA0019 gemeinsamer Primer
  source 1..27: mol_type = other DNA
ygagatctaggtgtcatcttctagtca

SEQ ID NO: 98 - DNA, 42 bp, synthetic construct
  misc_feature 1..42: note = MA0020 Primer Allel X
  source 1..42: mol_type = other DNA
gaaggtgaccaagttcatgctttgccagcatctctctgctcc

SEQ ID NO: 99 - DNA, 46 bp, synthetic construct
  misc_feature 1..46: note = MA0020 Primer Allel Y
  source 1..46: mol_type = other DNA
gaaggtcggagtcaacggattaattttgccagcatctctctgctca

SEQ ID NO: 100 - DNA, 25 bp, synthetic construct
  misc_feature 1..25: note = MA0020 gemeinsamer Primer
  source 1..25: mol_type = other DNA
gtgaatcggagaccaaggattgctt

SEQ ID NO: 101 - DNA, 45 bp, synthetic construct
  misc_feature 1..45: note = PZE-108095998 Primer Allel X
  source 1..45: mol_type = other DNA
gaaggtgaccaagttcatgcttcaaacaagcaagaggagcagcat

SEQ ID NO: 102 - DNA, 44 bp, synthetic construct
  misc_feature 1..44: note = PZE-108095998 Primer Allel Y
  source 1..44: mol_type = other DNA
gaaggtcggagtcaacggattcaaacaagcaagaggagcagcag

SEQ ID NO: 103 - DNA, 25 bp, synthetic construct
  misc_feature 1..25: note = PZE-108095998 gemeinsamer Primer
  source 1..25: mol_type = other DNA
ttgtctcggttgttaggtcgccaat

SEQ ID NO: 104 - DNA, 45 bp, synthetic construct
  misc_feature 1..45: note = PZE-108096011 Primer Allel X
  source 1..45: mol_type = other DNA
gaaggtgaccaagttcatgctccactaatgcagagatggagacta

SEQ ID NO: 105 - DNA, 44 bp, synthetic construct
  misc_feature 1..44: note = PZE-108096011 Primer Allel Y
  source 1..44: mol_type = other DNA
gaaggtcggagtcaacggattcactaatgcagagatggagactg

SEQ ID NO: 106 - DNA, 26 bp, synthetic construct
  misc_feature 1..26: note = PZE-108096011 gemeinsamer Primer
  source 1..26: mol_type = other DNA
catttacacactttgcaagggcccta

SEQ ID NO: 107 - DNA, 44 bp, synthetic construct
  misc_feature 1..44: note = PZE-108096791 Primer Allel X
  source 1..44: mol_type = other DNA
gaaggtgaccaagttcatgctagcacgaatcagcttccaagagt

SEQ ID NO: 108 - DNA, 43 bp, synthetic construct
  misc_feature 1..43: note = PZE-108096791 Primer Allel Y
  source 1..43: mol_type = other DNA
gaaggtcggagtcaacggattgcacgaatcagcttccaagagc

SEQ ID NO: 109 - DNA, 29 bp, synthetic construct
  misc_feature 1..29: note = PZE-108096791 gemeinsamer Primer
  source 1..29: mol_type = other DNA
attcgaagtgcactgcattctttgtcaaa

SEQ ID NO: 110 - DNA, 47 bp, synthetic construct
  misc_feature 1..47: note = PZE-108096791 Primer Allel X
  source 1..47: mol_type = other DNA
gaaggtgaccaagttcatgctgtcaaacatataagagggcaaagtca

SEQ ID NO: 111 - DNA, 47 bp, synthetic construct
  misc_feature 1..47: note = PZE-108096791 Primer Allel Y
  source 1..47: mol_type = other DNA
gaaggtcggagtcaacggattgtcaaacatataagagggcaaagtcg

SEQ ID NO: 112 - DNA, 29 bp, synthetic construct
  misc_feature 1..29: note = PZE-108096791 gemeinsamer Primer
  source 1..29: mol_type = other DNA
tgttccgttctacattttgatgtacctct

SEQ ID NO: 113 - DNA, 20 bp, synthetic construct
  misc_feature 1..20: note = bnlg1782 forward Primer
  source 1..20: mol_type = other DNA
cgatgctccgctaggaatag

SEQ ID NO: 114 - DNA, 20 bp, synthetic construct
  misc_feature 1..20: note = bnlg1782 reverse Primer
  source 1..20: mol_type = other DNA
tgtgttggaaattgacccaa

SEQ ID NO: 115 - DNA, 23 bp, synthetic construct
  misc_feature 1..23: note = umc1960 forward Primer
  source 1..23: mol_type = other DNA
ctgctggactacatggtggactt

SEQ ID NO: 116 - DNA, 21 bp, synthetic construct
  misc_feature 1..21: note = umc1960 reverse Primer
  source 1..21: mol_type = other DNA
gagctgtagcacccccaaaac

SEQ ID NO: 117 - DNA, 25 bp, synthetic construct
  misc_feature 1..25: note = bnlg240 forward Primer
  source 1..25: mol_type = other DNA
aagaacagaaggcattgatacataa

SEQ ID NO: 118 - DNA, 20 bp, synthetic construct
  misc_feature 1..20: note = bnlg240 reverse Primer
  source 1..20: mol_type = other DNA
tgcaggtgtatgggcagcta

SEQ ID NO: 119 - DNA, 24 bp, synthetic construct
  misc_feature 1..24: note = umc1121 forward Primer
  source 1..24: mol_type = other DNA
aaaacgacatgtcatcgtcttcaa

SEQ ID NO: 120 - DNA, 24 bp, synthetic construct
  misc_feature 1..24: note = umc1121 forward Primer
  source 1..24: mol_type = other DNA
ggggtcaggtacagggctagtagt

SEQ ID NO: 121 - DNA, 20 bp, synthetic construct
  misc_feature 1..20: note = bnlg1067 forward Primer
  source 1..20: mol_type = other DNA
ggcttgcttttgcttcactt

SEQ ID NO: 122 - DNA, 20 bp, synthetic construct
  misc_feature 1..20: note = bnlg1067 reverse Primer
  source 1..20: mol_type = other DNA
ctcatcccattcgttccact

SEQ ID NO: 123 - DNA, 42 bp, synthetic construct
  misc_feature 1..42: note = umc1287 forward Primer
  source 1..42: mol_type = other DNA
tgtaaaacgacggccagtatgggatgatcagtcgtttcagtc

SEQ ID NO: 124 - DNA, 24 bp, synthetic construct
  misc_feature 1..24: note = umc1287 reverse Primer
  source 1..24: mol_type = other DNA
aacgcacttcttgtagctgtaggg

SEQ ID NO: 125 - DNA, 20 bp, synthetic construct
  misc_feature 1..20: note = 579ZMPM0_2F Primer
  source 1..20: mol_type = other DNA
actcgcttgtctgtgtcacg

SEQ ID NO: 126 - DNA, 21 bp, synthetic construct
  misc_feature 1..21: note = 579ZMPM0_2R Primer
  source 1..21: mol_type = other DNA
cttgtcgattctccgatctca

SEQ ID NO: 127 - DNA, 20 bp, synthetic construct
  misc_feature 1..20: note = 579ZMPM0_4F Primer
  source 1..20: mol_type = other DNA
cttccagaccgacgtgagat

SEQ ID NO: 128 - DNA, 20 bp, synthetic construct
  misc_feature 1..20: note = 579ZMPM0_4R Primer
  source 1..20: mol_type = other DNA
aatactatgcaaggtcggcg

SEQ ID NO: 129 - DNA, 20 bp, synthetic construct
  misc_feature 1..20: note = 579ZMPM0_5F Primer
  source 1..20: mol_type = other DNA
ggcattattagctaggcgca

SEQ ID NO: 130 - DNA, 20 bp, synthetic construct
  misc_feature 1..20: note = 579ZMPM0_5R Primer
  source 1..20: mol_type = other DNA
ttgggaaactcaggttctgc

SEQ ID NO: 131 - DNA, 20 bp, synthetic construct
  misc_feature 1..20: note = 579ZMPM0_17F Primer
  source 1..20: mol_type = other DNA
tgtaccccagctacgacgtt

SEQ ID NO: 132 - DNA, 20 bp, synthetic construct
  misc_feature 1..20: note = 579ZMPM0_17R Primer
  source 1..20: mol_type = other DNA
aaccttcacgcaaagaatcg

SEQ ID NO: 133 - DNA, 20 bp, synthetic construct
  misc_feature 1..20: note = 579ZMPM0_16F Primer
  source 1..20: mol_type = other DNA
aaacatatgcgtgatcggct

SEQ ID NO: 134 - DNA, 20 bp, synthetic construct
  misc_feature 1..20: note = 579ZMPM0_16R Primer
  source 1..20: mol_type = other DNA
atggctcgtttcttcaggtg

SEQ ID NO: 135 - DNA, 22 bp, synthetic construct
  misc_feature 1..22: note = 579ZMPM0_25F Primer
  source 1..22: mol_type = other DNA
ttggaccaaacactatcgatcc

SEQ ID NO: 136 - DNA, 21 bp, synthetic construct
  misc_feature 1..21: note = 579ZMPM0_25R Primer
  source 1..21: mol_type = other DNA
cgttggcaaaacctaggaatc

SEQ ID NO: 137 - DNA, 20 bp, synthetic construct
  misc_feature 1..20: note = 579ZMPM0_22F Primer
  source 1..20: mol_type = other DNA
actggaactgcaggaaggtg

SEQ ID NO: 138 - DNA, 20 bp, synthetic construct
  misc_feature 1..20: note = 579ZMPM0_22R Primer
  source 1..20: mol_type = other DNA
gacgtttaaccggcagtcag

SEQ ID NO: 139 - DNA, 20 bp, synthetic construct
  misc_feature 1..20: note = 579ZMPM0_34F Primer
  source 1..20: mol_type = other DNA
tgaattgcaagcccacacta

SEQ ID NO: 140 - DNA, 20 bp, synthetic construct
  misc_feature 1..20: note = 579ZMPM0_34R Primer
  source 1..20: mol_type = other DNA
cctggtttgctgctcttcat

SEQ ID NO: 141 - DNA, 20 bp, synthetic construct
  misc_feature 1..20: note = 579ZMPM0_35F Primer
  source 1..20: mol_type = other DNA
ccaaatgaacacgaacacca

SEQ ID NO: 142 - DNA, 20 bp, synthetic construct
  misc_feature 1..20: note = 579ZMPM0_35R Primer
  source 1..20: mol_type = other DNA
ggcgtggtgactttttgtct

SEQ ID NO: 143 - DNA, 20 bp, synthetic construct
  misc_feature 1..20: note = 579ZMPM0_38F Primer
  source 1..20: mol_type = other DNA
cccaagatgaagatccgatg

SEQ ID NO: 144 - DNA, 20 bp, synthetic construct
  misc_feature 1..20: note = 579ZMPM0_38R Primer
  source 1..20: mol_type = other DNA
caaaccaaagaactcgagcg

SEQ ID NO: 145 - DNA, 20 bp, synthetic construct
  misc_feature 1..20: note = 579ZMPM0_37F Primer
  source 1..20: mol_type = other DNA
gtaatggggcagatgtttgg

SEQ ID NO: 146 - DNA, 20 bp, synthetic construct
  misc_feature 1..20: note = 579ZMPM0_37R Primer
  source 1..20: mol_type = other DNA
gcgactcttcgctacacacc

SEQ ID NO: 147 - DNA, 24 bp, synthetic construct
  misc_feature 1..24: note = 579ZMPM0_41F Primer
  misc_feature 1..3: note = n is a, c, g, or t
  source 1..24: mol_type = other DNA
nnnccctgttcatgtaacttcaat

SEQ ID NO: 148 - DNA, 20 bp, synthetic construct
  misc_feature 1..20: note = 579ZMPM0_41R Primer
  source 1..20: mol_type = other DNA
tgcacacgataaggacatgc

SEQ ID NO: 149 - DNA, 24 bp, synthetic construct
  misc_feature 1..24: note = 579ZMPM0_41F Primer
  misc_feature 1..3: note = n is a, c, g, or t
  source 1..24: mol_type = other DNA
nnnccctgttcatgtaacttcaat

SEQ ID NO: 150 - DNA, 20 bp, synthetic construct
  misc_feature 1..20: note = 579ZMPM0_41R Primer
  source 1..20: mol_type = other DNA
tgcacacgataaggacatgc

SEQ ID NO: 151 - DNA, 20 bp, synthetic construct
  misc_feature 1..20: note = 579ZMPM0_46F Primer
  source 1..20: mol_type = other DNA
tcaagagaactctgggtggc

SEQ ID NO: 152 - DNA, 20 bp, synthetic construct
  misc_feature 1..20: note = 579ZMPM0_46r Primer
  source 1..20: mol_type = other DNA
ggccaacaatgacgagagtc

SEQ ID NO: 153 - DNA, 20 bp, synthetic construct
  misc_feature 1..20: note = 579ZMPM0_180F Primer
  source 1..20: mol_type = other DNA
gggagggttgttctggtttt

SEQ ID NO: 154 - DNA, 20 bp, synthetic construct
  misc_feature 1..20: note = 579ZMPM0_180R2 Primer
  source 1..20: mol_type = other DNA
ggtccttgtcaatgtcaccc

SEQ ID NO: 155 - DNA, 20 bp, synthetic construct
  misc_feature 1..20: note = 579ZMPM0_48F Primer
  source 1..20: mol_type = other DNA
atggacccccgttgttatct

SEQ ID NO: 156 - DNA, 20 bp, synthetic construct
  misc_feature 1..20: note = 579ZMPM0_48R Primer
  source 1..20: mol_type = other DNA
gcctgcagacaaattcctgt

SEQ ID NO: 157 - DNA, 20 bp, synthetic construct
  misc_feature 1..20: note = 579ZMPM0_48F Primer
  source 1..20: mol_type = other DNA
atggacccccgttgttatct

SEQ ID NO: 158 - DNA, 20 bp, synthetic construct
  misc_feature 1..20: note = 579ZMPM0_48R Primer
  source 1..20: mol_type = other DNA
gcctgcagacaaattcctgt

SEQ ID NO: 159 - DNA, 20 bp, synthetic construct
  misc_feature 1..20: note = 579ZMPM0_56F Primer
  source 1..20: mol_type = other DNA
cctgtcatggtgggaacaat

SEQ ID NO: 160 - DNA, 20 bp, synthetic construct
  misc_feature 1..20: note = 579ZMPM0_56R Primer
  source 1..20: mol_type = other DNA
ctcatcagcgaagcgaaaaa

SEQ ID NO: 161 - DNA, 20 bp, synthetic construct
  misc_feature 1..20: note = 579ZMPM0_51F Primer
  source 1..20: mol_type = other DNA
accctctccttgctattggc

SEQ ID NO: 162 - DNA, 20 bp, synthetic construct
  misc_feature 1..20: note = 579ZMPM0_51R Primer
  source 1..20: mol_type = other DNA
ctccagctcttcgttcgttc

SEQ ID NO: 163 - DNA, 20 bp, synthetic construct
  misc_feature 1..20: note = 579ZMPM0_199F Primer
  source 1..20: mol_type = other DNA
gcaggctggacaaaagtgtt

SEQ ID NO: 164 - DNA, 20 bp, synthetic construct
  misc_feature 1..20: note = 579ZMPM0_199R Primer
  source 1..20: mol_type = other DNA
ttctttttgcggcctatctg

SEQ ID NO: 165 - DNA, 20 bp, synthetic construct
  misc_feature 1..20: note = 579ZMPM0_63F Primer
  source 1..20: mol_type = other DNA
atttgcttggcgtaatcctg

SEQ ID NO: 166 - DNA, 20 bp, synthetic construct
  misc_feature 1..20: note = 579ZMPM0_63R Primer
  source 1..20: mol_type = other DNA
cagccgtgtttttctttgct

SEQ ID NO: 167 - DNA, 20 bp, synthetic construct
  misc_feature 1..20: note = 579ZMPM0_208F Primer
  source 1..20: mol_type = other DNA
cgcacggatcaagaagagtt

SEQ ID NO: 168 - DNA, 20 bp, synthetic construct
  misc_feature 1..20: note = 579ZMPM0_208R Primer
  source 1..20: mol_type = other DNA
caatcgccatgcatactttg

SEQ ID NO: 169 - DNA, 22 bp, synthetic construct
  misc_feature 1..22: note = 579ZMPM0_206F Primer
  source 1..22: mol_type = other DNA
atggtacaagtgtcgatccctc

SEQ ID NO: 170 - DNA, 20 bp, synthetic construct
  misc_feature 1..20: note = 579ZMPM0_206R Primer
  source 1..20: mol_type = other DNA
aatgaatcgatgtcgctggt

SEQ ID NO: 171 - DNA, 22 bp, synthetic construct
  misc_feature 1..22: note = 579ZMPM0_86F Primer
  source 1..22: mol_type = other DNA
cacaactaaagaggaaaccgga

SEQ ID NO: 172 - DNA, 20 bp, synthetic construct
  misc_feature 1..20: note = 579ZMPM0_86R Primer
  source 1..20: mol_type = other DNA
ggctgacggtctagtcttcg

SEQ ID NO: 173 - DNA, 20 bp, synthetic construct
  misc_feature 1..20: note = 579ZMPM0_79F Primer
  source 1..20: mol_type = other DNA
aaccaaatggggtcttagcc

SEQ ID NO: 174 - DNA, 20 bp, synthetic construct
  misc_feature 1..20: note = 579ZMPM0_79R Primer
  source 1..20: mol_type = other DNA
atccgccactggtcaaaata

SEQ ID NO: 175 - DNA, 20 bp, synthetic construct
  misc_feature 1..20: note = 579ZMPM0_278F Primer
  source 1..20: mol_type = other DNA
catcgcaacatcagcaacat

SEQ ID NO: 176 - DNA, 20 bp, synthetic construct
  misc_feature 1..20: note = 579ZMPM0_278R Primer
  source 1..20: mol_type = other DNA
acgtttgttcccttcatcca

SEQ ID NO: 177 - DNA, 20 bp, synthetic construct
  misc_feature 1..20: note = 579zmpm0_209F Primer
  source 1..20: mol_type = other DNA
ctgtgcttctggtgctgaaa

SEQ ID NO: 178 - DNA, 20 bp, synthetic construct
  misc_feature 1..20: note = 579zmpm0_209R Primer
  source 1..20: mol_type = other DNA
ctttcccgcctgtaaatgaa

SEQ ID NO: 179 - DNA, 22 bp, synthetic construct
  misc_feature 1..22: note = 579zmpm0_86F Primer
  source 1..22: mol_type = other DNA
cacaactaaagaggaaaccgga

SEQ ID NO: 180 - DNA, 22 bp, synthetic construct
  misc_feature 1..22: note = 579zmpm0_86F
  source 1..22: mol_type = other DNA
cacaactaaagaggaaaccgga

SEQ ID NO: 181 - DNA, 20 bp, synthetic construct
  misc_feature 1..20: note = 579zmpm0_87F Primer
  source 1..20: mol_type = other DNA
ctcaccccaccctaccctat

SEQ ID NO: 182 - DNA, 20 bp, synthetic construct
  misc_feature 1..20: note = 579zmpm0_87R Primer
  source 1..20: mol_type = other DNA
ggggagctgttgaaggaaat

SEQ ID NO: 183 - DNA, 20 bp, synthetic construct
  misc_feature 1..20: note = 579zmpm0_91F Primer
  source 1..20: mol_type = other DNA
acgtcgatctgcttgctacc

SEQ ID NO: 184 - DNA, 20 bp, synthetic construct
  misc_feature 1..20: note = 579zmpm0_91R Primer
  source 1..20: mol_type = other DNA
gagacctagcgatccaacga

SEQ ID NO: 185 - DNA, 21 bp, synthetic construct
  misc_feature 1..21: note = 579zmpm0_216F Primer
  source 1..21: mol_type = other DNA
ctccatagtgtttcggccttt

SEQ ID NO: 186 - DNA, 20 bp, synthetic construct
  misc_feature 1..20: note = 579zmpm0_216R Primer
  source 1..20: mol_type = other DNA
gccctcaggacttaccgact

SEQ ID NO: 187 - DNA, 20 bp, synthetic construct
  misc_feature 1..20: note = 579ZMPM0_95F Primer
  source 1..20: mol_type = other DNA
gtcactatacggagacggcg

SEQ ID NO: 188 - DNA, 20 bp, synthetic construct
  misc_feature 1..20: note = 579ZMPM0_95R Primer
  source 1..20: mol_type = other DNA
ctcggccttcaatttgtgat

SEQ ID NO: 189 - DNA, 20 bp, synthetic construct
  misc_feature 1..20: note = 579ZMPM0_99F Primer
  source 1..20: mol_type = other DNA
agagcaacatgccttgaacc

SEQ ID NO: 190 - DNA, 20 bp, synthetic construct
  misc_feature 1..20: note = 579ZMPM0_99R Primer
  source 1..20: mol_type = other DNA
gttttgatcccgaagccttt

SEQ ID NO: 191 - DNA, 21 bp, synthetic construct
  misc_feature 1..21: note = 579ZMPM0_244F Primer
  source 1..21: mol_type = other DNA
attcaatggacacgcaacaat

SEQ ID NO: 192 - DNA, 20 bp, synthetic construct
  misc_feature 1..20: note = 579ZMPM0_244R Primer
  source 1..20: mol_type = other DNA
tgtggtggggattttagtgg

SEQ ID NO: 193 - DNA, 20 bp, synthetic construct
  misc_feature 1..20: note = 579ZMPM0_241F Primer
  source 1..20: mol_type = other DNA
cattcgaaaatctggccact

SEQ ID NO: 194 - DNA, 20 bp, synthetic construct
  misc_feature 1..20: note = 579ZMPM0_241R Primer
  source 1..20: mol_type = other DNA
gccaatggaatggagaacag

SEQ ID NO: 195 - DNA, 20 bp, synthetic construct
  misc_feature 1..20: note = 579ZMPM0_109F Primer
  source 1..20: mol_type = other DNA
gagcaaatcagatgcagcaa

SEQ ID NO: 196 - DNA, 20 bp, synthetic construct
  misc_feature 1..20: note = 579ZMPM0_109R Primer
  source 1..20: mol_type = other DNA
tgatgatggtctgttgccag

SEQ ID NO: 197 - DNA, 20 bp, synthetic construct
  misc_feature 1..20: note = 579ZMPM0_109F Primer
  source 1..20: mol_type = other DNA
gagcaaatcagatgcagcaa

SEQ ID NO: 198 - DNA, 20 bp, synthetic construct
  misc_feature 1..20: note = 579ZMPM0_109R Primer
  source 1..20: mol_type = other DNA
tgatgatggtctgttgccag

SEQ ID NO: 199 - DNA, 20 bp, synthetic construct
  misc_feature 1..20: note = 579ZMPM0_247F Primer
  source 1..20: mol_type = other DNA
tgcaaccatatgttgatggg

SEQ ID NO: 200 - DNA, 20 bp, synthetic construct
  misc_feature 1..20: note = 579ZMPM0_247R Primer
  source 1..20: mol_type = other DNA
cagcttgagacaaacgctga

SEQ ID NO: 201 - DNA, 20 bp, synthetic construct
  misc_feature 1..20: note = 579ZMPM0_112F Primer
  source 1..20: mol_type = other DNA
tgaaaaccctacctgaagcg

SEQ ID NO: 202 - DNA, 20 bp, synthetic construct
  misc_feature 1..20: note = 579ZMPM0_112R Primer
  source 1..20: mol_type = other DNA
actgcactgatccggacttc

SEQ ID NO: 203 - DNA, 21 bp, synthetic construct
  misc_feature 1..21: note = 579ZMPM0_125F Primer
  source 1..21: mol_type = other DNA
tcgaggctaacatggtctctg

SEQ ID NO: 204 - DNA, 21 bp, synthetic construct
  misc_feature 1..21: note = 579ZMPM0_125R
  source 1..21: mol_type = other DNA
catacacttcatgtcgtcccg

SEQ ID NO: 205 - DNA, 20 bp, synthetic construct
  misc_feature 1..20: note = 579ZMPM0_253F Primer
  source 1..20: mol_type = other DNA
ggccgggacgtactagtgta

SEQ ID NO: 206 - DNA, 20 bp, synthetic construct
  misc_feature 1..20: note = 579ZMPM0_253R Primer
  source 1..20: mol_type = other DNA
tggttgtcatcatttggcac

SEQ ID NO: 207 - DNA, 21 bp, synthetic construct
  misc_feature 1..21: note = 579ZMPM0_125F Primer
  source 1..21: mol_type = other DNA
tcgaggctaacatggtctctg

SEQ ID NO: 208 - DNA, 21 bp, synthetic construct
  misc_feature 1..21: note = 579ZMPM0_125R Primer
  source 1..21: mol_type = other DNA
catacacttcatgtcgtcccg

SEQ ID NO: 209 - DNA, 20 bp, synthetic construct
  misc_feature 1..20: note = 579ZMPM0_128F Primer
  source 1..20: mol_type = other DNA
gctcaaggcgatacatgctt

SEQ ID NO: 210 - DNA, 20 bp, synthetic construct
  misc_feature 1..20: note = 579ZMPM0_128F
  source 1..20: mol_type = other DNA
gctcaaggcgatacatgctt

SEQ ID NO: 211 - DNA, 16 bp, synthetic construct
  misc_feature 1..16: note = 579ZMPM0_136F Primer
  source 1..16: mol_type = other DNA
ggcttgactgtaatgg

SEQ ID NO: 212 - DNA, 20 bp, synthetic construct
  misc_feature 1..20: note = 579ZMPM0_136R Primer
  source 1..20: mol_type = other DNA
tttctgctcacacttcggtg

SEQ ID NO: 213 - DNA, 25 bp, synthetic construct
  misc_feature 1..25: note = 579ZMPM0_131F Primer
  source 1..25: mol_type = other DNA
tcaagcaaacgagactcttcttgta

SEQ ID NO: 214 - DNA, 20 bp, synthetic construct
  misc_feature 1..20: note = 579ZMPM0_131R Primer
  source 1..20: mol_type = other DNA
tagccatggacagatcgaca

SEQ ID NO: 215 - DNA, 20 bp, synthetic construct
  misc_feature 1..20: note = 579ZMPM0_137F Primer
  source 1..20: mol_type = other DNA
cggaccttgtactccgtcac

SEQ ID NO: 216 - DNA, 20 bp, synthetic construct
  misc_feature 1..20: note = 579ZMPM0_137R Primer
  source 1..20: mol_type = other DNA
agaatgtggaggctacggtg

SEQ ID NO: 217 - DNA, 20 bp, synthetic construct
  misc_feature 1..20: note = 579ZMPM0_138F Primer
  source 1..20: mol_type = other DNA
tgaaatttaggacttgcccg

SEQ ID NO: 218 - DNA, 20 bp, synthetic construct
  misc_feature 1..20: note = 579ZMPM0_138R Primer
  source 1..20: mol_type = other DNA
acatctgaacaccgcattga

SEQ ID NO: 219 - DNA, 20 bp, synthetic construct
  misc_feature 1..20: note = 579ZMPM0_147F Primer
  source 1..20: mol_type = other DNA
cttgtggtcccactccactt

SEQ ID NO: 220 - DNA, 20 bp, synthetic construct
  misc_feature 1..20: note = 579ZMPM0_147R Primer
  source 1..20: mol_type = other DNA
ttactttccatggcctccaa

SEQ ID NO: 221 - DNA, 20 bp, synthetic construct
  misc_feature 1..20: note = 579ZMPM0_145F Primer
  source 1..20: mol_type = other DNA
tgtgctcgggtattgacgta

SEQ ID NO: 222 - DNA, 20 bp, synthetic construct
  misc_feature 1..20: note = 579ZMPM0_145R Primer
  source 1..20: mol_type = other DNA
ccgtcaacttcctcccctat

SEQ ID NO: 223 - DNA, 20 bp, synthetic construct
  misc_feature 1..20: note = 579ZMPM0_262F Primer
  source 1..20: mol_type = other DNA
ttgctggcttgttatcctcc

SEQ ID NO: 224 - DNA, 20 bp, synthetic construct
  misc_feature 1..20: note = 579ZMPM0_262R Primer
  source 1..20: mol_type = other DNA
ccctgtcgttcaaggaaaaa

SEQ ID NO: 225 - DNA, 20 bp, synthetic construct
  misc_feature 1..20: note = 579ZMPM0_161F Primer
  source 1..20: mol_type = other DNA
taggtaacagaattgcgggc

SEQ ID NO: 226 - DNA, 20 bp, synthetic construct
  misc_feature 1..20: note = 579ZMPM0_161R Primer
  source 1..20: mol_type = other DNA
tttctaaggcatgggagtgc

SEQ ID NO: 227 - DNA, 20 bp, synthetic construct
  misc_feature 1..20: note = 579ZMPM0_265F Primer
  source 1..20: mol_type = other DNA
catttcatggcatatgagcg

SEQ ID NO: 228 - DNA, 20 bp, synthetic construct
  misc_feature 1..20: note = 579ZMPM0_265R Primer
  source 1..20: mol_type = other DNA
ctaaaggccctgttcccagt

SEQ ID NO: 229 - DNA, 20 bp, synthetic construct
  misc_feature 1..20: note = ZNF1_GH034_F_Primer
  source 1..20: mol_type = other DNA
tggttggtgtcgaagctgag

SEQ ID NO: 230 - DNA, 20 bp, synthetic construct
  misc_feature 1..20: note = ZNF1_GH033_R_Primer
  source 1..20: mol_type = other DNA
atttatcccggcctttgcat

SEQ ID NO: 231 - DNA, 22 bp, synthetic construct
  misc_feature 1..22: note = HYD_GH039_F_Primer
  source 1..22: mol_type = other DNA
gatctacagggaagcccactga

SEQ ID NO: 232 - DNA, 25 bp, synthetic construct
  misc_feature 1..25: note = HYD_GH040_R_Primer
  source 1..25: mol_type = other DNA
tttttccttgaggcagttatatgct

SEQ ID NO: 233 - DNA, 17 bp, synthetic construct
  misc_feature 1..17: note = RLK4_GH220_F_Primer
  source 1..17: mol_type = other DNA
ttgtgcagcggagggaa

SEQ ID NO: 234 - DNA, 19 bp, synthetic construct
  misc_feature 1..19: note = RLK4_GH221_R_Primer
  source 1..19: mol_type = other DNA
ccagggcaccagcaagaat

SEQ ID NO: 235 - DNA, 19 bp, synthetic construct
  misc_feature 1..19: note = EXT1_GH168_F_Primer
  source 1..19: mol_type = other DNA
cgactacaagacgcgtacc

SEQ ID NO: 236 - DNA, 19 bp, synthetic construct
  misc_feature 1..19: note = EXT1_GH170_R_Primer
  source 1..19: mol_type = other DNA
ggtgtcgatggtgaggttc

SEQ ID NO: 237 - DNA, 20 bp, synthetic construct
  misc_feature 1..20: note = RLK1_GH138_F_Primer
  source 1..20: mol_type = other DNA
tattgttggtgctgttgccg

SEQ ID NO: 238 - DNA, 20 bp, synthetic construct
  misc_feature 1..20: note = RLK1_GH139_R_Primer
  source 1..20: mol_type = other DNA
ggactcaatccttgtccctg

SEQ ID NO: 239 - DNA, 20 bp, synthetic construct
  misc_feature 1..20: note = RET1_GH055_F_Primer
  source 1..20: mol_type = other DNA
cgctcgtttgccagatagcc

SEQ ID NO: 240 - DNA, 20 bp, synthetic construct
  misc_feature 1..20: note = RET1_GH056_R_Primer
  source 1..20: mol_type = other DNA
cacggtgtgtgccagtttgt

SEQ ID NO: 241 - DNA, 42 bp, synthetic construct
  misc_feature 1..42: note = MA0021 Primer Allel X
  source 1..42: mol_type = other DNA
gaaggtgaccaagttcatgctgagctcatctcgtccaagccc

SEQ ID NO: 242 - DNA, 42 bp, synthetic construct
  misc_feature 1..42: note = MA0021 Primer Allel Y
  source 1..42: mol_type = other DNA
gaaggtcggagtcaacggattgagctcatctcgtccaagccg

SEQ ID NO: 243 - DNA, 19 bp, synthetic construct
  misc_feature 1..19: note = MA0021 gemeinsamer Primer
  source 1..19: mol_type = other DNA
cgctgcggtgccgggtgat

SEQ ID NO: 244 - DNA, 47 bp, synthetic construct
  misc_feature 1..47: note = MA0022 Primer Allel X
  source 1..47: mol_type = other DNA
gaaggtgaccaagttcatgctcaccaacacaatagtcgtccaaatgt

SEQ ID NO: 245 - DNA, 46 bp, synthetic construct
  misc_feature 1..46: note = MA0022 Primer Allel Y
  source 1..46: mol_type = other DNA
gaaggtcggagtcaacggattaccaacacaatagtcgtccaaatgc

SEQ ID NO: 246 - DNA, 25 bp, synthetic construct
  misc_feature 1..25: note = MA0022 gemeinsamer Primer
  source 1..25: mol_type = other DNA
cagccaatatttccctcagtggctt

SEQ ID NO: 247 - DNA, 24 bp, synthetic construct
  misc_feature 1..24: note = MA04916-6f Primer
  source 1..24: mol_type = other DNA
tgtttcaggaatcacgcaactgga

SEQ ID NO: 248 - DNA, 22 bp, synthetic construct
  misc_feature 1..22: note = MA04916-6r Primer
  source 1..22: mol_type = other DNA
gcaccacgccatgaccaacatc

SEQ ID NO: 249 - DNA, 22 bp, synthetic construct
  misc_feature 1..22: note = TG10013-10.f Primer
  source 1..22: mol_type = other DNA
cttcctacagaagaacgagagt

SEQ ID NO: 250 - DNA, 21 bp, synthetic construct
  misc_feature 1..21: note = TG10013-11.r Primer
  source 1..21: mol_type = other DNA
ttcctcacgagctctgtggtc